European Patent Application EP 4 130 263 A1, published February 8, 2023. Title: Compound and method for an editing of the HAX1 gene. Applicant: Eberhard Karls Universität Tübingen - Medizinische Fakultät. The sequence listing filed with the application follows.

SEQUENCE LISTING (565 sequences)

SEQ ID NO: 1 - DNA, 20 bp, artificial sequence
  sgRNA
aggtcttcctcaaatttgaa

SEQ ID NO: 2 - DNA, 20 bp, artificial sequence
  sgRNA
gataaagcctttcaaatttg

SEQ ID NO: 3 - DNA, 20 bp, artificial sequence
  sgRNA
tcaaatttgaggaagacctt

SEQ ID NO: 4 - DNA, 20 bp, artificial sequence
  sgRNA
tgaaatggaggcgggaccga

SEQ ID NO: 5 - DNA, 20 bp, artificial sequence
  sgRNA
gccggacgtgaaatggaggc

SEQ ID NO: 6 - DNA, 20 bp, artificial sequence
  sgRNA
agccggacgtgaaatggagg

SEQ ID NO: 7 - DNA, 20 bp, artificial sequence
  sgRNA
gtaagccggacgtgaaatgg

SEQ ID NO: 8 - DNA, 20 bp, artificial sequence
  sgRNA
acggtaagccggacgtgaaa

SEQ ID NO: 9 - DNA, 20 bp, artificial sequence
  sgRNA
tcccgcctccatttcacgtc

SEQ ID NO: 10 - DNA, 20 bp, artificial sequence
  sgRNA
tgtcgtaaacgacggtaagc

SEQ ID NO: 11 - DNA, 20 bp, artificial sequence
  sgRNA
cctgacactgtcgtaaacga

SEQ ID NO: 12 - DNA, 20 bp, artificial sequence
  sgRNA
ccgtcgtttacgacagtgtc

SEQ ID NO: 13 - DNA, 20 bp, artificial sequence
  sgRNA
ttacgacagtgtcaggatcg

SEQ ID NO: 14 - DNA, 20 bp, artificial sequence
  sgRNA
tacgacagtgtcaggatcgc

SEQ ID NO: 15 - DNA, 20 bp, artificial sequence
  sgRNA
aggatcgcgggcttgctttc

SEQ ID NO: 16 - DNA, 20 bp, artificial sequence
  sgRNA
gggcttgctttccggtagcg

SEQ ID NO: 17 - DNA, 20 bp, artificial sequence
  sgRNA
gaggcgtcagcccacgctac

SEQ ID NO: 18 - DNA, 20 bp, artificial sequence
  sgRNA
ggcttgctttccggtagcgt

SEQ ID NO: 19 - DNA, 20 bp, artificial sequence
  sgRNA
gccctgtgagaaattgagcg

SEQ ID NO: 20 - DNA, 20 bp, artificial sequence
  sgRNA
cgcctcgctcaatttctcac

SEQ ID NO: 21 - DNA, 20 bp, artificial sequence
  sgRNA
gcctcgctcaatttctcaca

SEQ ID NO: 22 - DNA, 20 bp, artificial sequence
  sgRNA
aatttctcacagggctgcgc

SEQ ID NO: 23 - DNA, 20 bp, artificial sequence
  sgRNA
agtggtccattcgcagacgg

SEQ ID NO: 24 - DNA, 20 bp, artificial sequence
  sgRNA
cagtggtccattcgcagacg

SEQ ID NO: 25 - DNA, 20 bp, artificial sequence
  sgRNA
ccagtggtccattcgcagac

SEQ ID NO: 26 - DNA, 20 bp, artificial sequence
  sgRNA
tccagtggtccattcgcaga

SEQ ID NO: 27 - DNA, 20 bp, artificial sequence
  sgRNA
aggtttcccccgtctgcgaa

SEQ ID NO: 28 - DNA, 20 bp, artificial sequence
  sgRNA
cccgtctgcgaatggaccac

SEQ ID NO: 29 - DNA, 20 bp, artificial sequence
  sgRNA
gtctgcgaatggaccactgg

SEQ ID NO: 30 - DNA, 20 bp, artificial sequence
  sgRNA
tctgcgaatggaccactgga

SEQ ID NO: 31 - DNA, 20 bp, artificial sequence
  sgRNA
ctgcgaatggaccactggag

SEQ ID NO: 32 - DNA, 20 bp, artificial sequence
  sgRNA
gaacctttgaacccctccag

SEQ ID NO: 33 - DNA, 20 bp, artificial sequence
  sgRNA
ggaccactggaggggttcaa

SEQ ID NO: 34 - DNA, 20 bp, artificial sequence
  sgRNA
caaaggttcgcgtcccagta

SEQ ID NO: 35 - DNA, 20 bp, artificial sequence
  sgRNA
aaaggttcgcgtcccagtac

SEQ ID NO: 36 - DNA, 20 bp, artificial sequence
  sgRNA
aagaggctcattcccgtact

SEQ ID NO: 37 - DNA, 20 bp, artificial sequence
  sgRNA
aaagaggctcattcccgtac

SEQ ID NO: 38 - DNA, 20 bp, artificial sequence
  sgRNA
agccccggaagagatcaaag

SEQ ID NO: 39 - DNA, 20 bp, artificial sequence
  sgRNA
tgagcctctttgatctcttc

SEQ ID NO: 40 - DNA, 20 bp, artificial sequence
  sgRNA
gagcctctttgatctcttcc

SEQ ID NO: 41 - DNA, 20 bp, artificial sequence
  sgRNA
agcctctttgatctcttccg

SEQ ID NO: 42 - DNA, 20 bp, artificial sequence
  sgRNA
caggaaagccgaaaaagccc

SEQ ID NO: 43 - DNA, 20 bp, artificial sequence
  sgRNA
gatctcttccggggcttttt

SEQ ID NO: 44 - DNA, 20 bp, artificial sequence
  sgRNA
cggggctttttcggctttcc

SEQ ID NO: 45 - DNA, 20 bp, artificial sequence
  sgRNA
ttttcggctttcctggacct

SEQ ID NO: 46 - DNA, 20 bp, artificial sequence
  sgRNA
tactctcacctccgaggtcc

SEQ ID NO: 47 - DNA, 20 bp, artificial sequence
  sgRNA
tcggctttcctggacctcgg

SEQ ID NO: 48 - DNA, 20 bp, artificial sequence
  sgRNA
cggacctactctcacctccg

SEQ ID NO: 49 - DNA, 20 bp, artificial sequence
  sgRNA
tggacctcggaggtgagagt

SEQ ID NO: 50 - DNA, 20 bp, artificial sequence
  sgRNA
ctcggaggtgagagtaggtc

SEQ ID NO: 51 - DNA, 20 bp, artificial sequence
  sgRNA
aggtgagagtaggtccggct

SEQ ID NO: 52 - DNA, 20 bp, artificial sequence
  sgRNA
acccccacccttgtccgagc

SEQ ID NO: 53 - DNA, 20 bp, artificial sequence
  sgRNA
gagtaggtccggctcggaca

SEQ ID NO: 54 - DNA, 20 bp, artificial sequence
  sgRNA
agtaggtccggctcggacaa

SEQ ID NO: 55 - DNA, 20 bp, artificial sequence
  sgRNA
aggtccggctcggacaaggg

SEQ ID NO: 56 - DNA, 20 bp, artificial sequence
  sgRNA
ggtccggctcggacaagggt

SEQ ID NO: 57 - DNA, 20 bp, artificial sequence
  sgRNA
gtccggctcggacaagggtg

SEQ ID NO: 58 - DNA, 20 bp, artificial sequence
  sgRNA
tccggctcggacaagggtgg

SEQ ID NO: 59 - DNA, 20 bp, artificial sequence
  sgRNA
acaagggtgggggtcgtctg

SEQ ID NO: 60 - DNA, 20 bp, artificial sequence
  sgRNA
caagggtgggggtcgtctga

SEQ ID NO: 61 - DNA, 20 bp, artificial sequence
  sgRNA
aagggtgggggtcgtctgag

SEQ ID NO: 62 - DNA, 20 bp, artificial sequence
  sgRNA
tttccaaaaataagacgtag

SEQ ID NO: 63 - DNA, 20 bp, artificial sequence
  sgRNA
ttttccaaaaataagacgta

SEQ ID NO: 64 - DNA, 20 bp, artificial sequence
  sgRNA
tttttccaaaaataagacgt

SEQ ID NO: 65 - DNA, 20 bp, artificial sequence
  sgRNA
tgacccctacgtcttatttt

SEQ ID NO: 66 - DNA, 20 bp, artificial sequence
  sgRNA
gagttgaaggagtgggacag

SEQ ID NO: 67 - DNA, 20 bp, artificial sequence
  sgRNA
tctgcaggagttgaaggagt

SEQ ID NO: 68 - DNA, 20 bp, artificial sequence
  sgRNA
ctctgcaggagttgaaggag

SEQ ID NO: 69 - DNA, 20 bp, artificial sequence
  sgRNA
gtcctctctgcaggagttga

SEQ ID NO: 70 - DNA, 20 bp, artificial sequence
  sgRNA
ctccttcaactcctgcagag

SEQ ID NO: 71 - DNA, 20 bp, artificial sequence
  sgRNA
gcgacttctgtcctctctgc

SEQ ID NO: 72 - DNA, 20 bp, artificial sequence
  sgRNA
ccgccttggttactgtggcg

SEQ ID NO: 73 - DNA, 20 bp, artificial sequence
  sgRNA
accgccttggttactgtggc

SEQ ID NO: 74 - DNA, 20 bp, artificial sequence
  sgRNA
gaccgccttggttactgtgg

SEQ ID NO: 75 - DNA, 20 bp, artificial sequence
  sgRNA
aatgaccgccttggttactg

SEQ ID NO: 76 - DNA, 20 bp, artificial sequence
  sgRNA
tcaccccgccacagtaacca

SEQ ID NO: 77 - DNA, 20 bp, artificial sequence
  sgRNA
ccccgccacagtaaccaagg

SEQ ID NO: 78 - DNA, 20 bp, artificial sequence
  sgRNA
tctcctcttaatgaccgcct

SEQ ID NO: 79 - DNA, 20 bp, artificial sequence
  sgRNA
taaccaaggcggtcattaag

SEQ ID NO: 80 - DNA, 20 bp, artificial sequence
  sgRNA
catcaccccaggttggagaa

SEQ ID NO: 81 - DNA, 20 bp, artificial sequence
  sgRNA
aactaagcctttctccaacc

SEQ ID NO: 82 - DNA, 20 bp, artificial sequence
  sgRNA
actaagcctttctccaacct

SEQ ID NO: 83 - DNA, 20 bp, artificial sequence
  sgRNA
ctaagcctttctccaacctg

SEQ ID NO: 84 - DNA, 20 bp, artificial sequence
  sgRNA
cctgttgcatcaccccaggt

SEQ ID NO: 85 - DNA, 20 bp, artificial sequence
  sgRNA
ggtccctgttgcatcacccc

SEQ ID NO: 86 - DNA, 20 bp, artificial sequence
  sgRNA
ccaacctggggtgatgcaac

SEQ ID NO: 87 - DNA, 20 bp, artificial sequence
  sgRNA
caacctggggtgatgcaaca

SEQ ID NO: 88 - DNA, 20 bp, artificial sequence
  sgRNA
ggggtgatgcaacagggacc

SEQ ID NO: 89 - DNA, 20 bp, artificial sequence
  sgRNA
gggtgatgcaacagggaccc

SEQ ID NO: 90 - DNA, 20 bp, artificial sequence
  sgRNA
tgatgcaacagggacccggg

SEQ ID NO: 91 - DNA, 20 bp, artificial sequence
  sgRNA
gatgcaacagggacccgggc

SEQ ID NO: 92 - DNA, 20 bp, artificial sequence
  sgRNA
atgcaacagggacccgggcg

SEQ ID NO: 93 - DNA, 20 bp, artificial sequence
  sgRNA
cctcacggtcttccccgccc

SEQ ID NO: 94 - DNA, 20 bp, artificial sequence
  sgRNA
ccctcacggtcttccccgcc

SEQ ID NO: 95 - DNA, 20 bp, artificial sequence
  sgRNA
cccgggcggggaagaccgtg

SEQ ID NO: 96 - DNA, 20 bp, artificial sequence
  sgRNA
ccgggcggggaagaccgtga

SEQ ID NO: 97 - DNA, 20 bp, artificial sequence
  sgRNA
tcttattccccagaccctca

SEQ ID NO: 98 - DNA, 20 bp, artificial sequence
  sgRNA
cggggaagaccgtgagggtc

SEQ ID NO: 99 - DNA, 20 bp, artificial sequence
  sgRNA
ggggaagaccgtgagggtct

SEQ ID NO: 100 - DNA, 20 bp, artificial sequence
  sgRNA
gggaagaccgtgagggtctg

SEQ ID NO: 101 - DNA, 20 bp, artificial sequence
  sgRNA
aagacagtgagcaagtgagc

SEQ ID NO: 102 - DNA, 20 bp, artificial sequence
  sgRNA
tgagcaagtgagcaggacct

SEQ ID NO: 103 - DNA, 20 bp, artificial sequence
  sgRNA
gagcaagtgagcaggacctt

SEQ ID NO: 104 - DNA, 20 bp, artificial sequence
  sgRNA
agtccctcctctctctccca

SEQ ID NO: 105 - DNA, 20 bp, artificial sequence
  sgRNA
agcaggaccttgggagagag

SEQ ID NO: 106 - DNA, 20 bp, artificial sequence
  sgRNA
aggaccttgggagagagagg

SEQ ID NO: 107 - DNA, 20 bp, artificial sequence
  sgRNA
ggaccttgggagagagagga

SEQ ID NO: 108 - DNA, 20 bp, artificial sequence
  sgRNA
ttgggagagagaggagggac

SEQ ID NO: 109 - DNA, 20 bp, artificial sequence
  sgRNA
tgggagagagaggagggact

SEQ ID NO: 110 - DNA, 20 bp, artificial sequence
  sgRNA
gggagagagaggagggactg

SEQ ID NO: 111 - DNA, 20 bp, artificial sequence
  sgRNA
ggggcacactgaagaaaaac

SEQ ID NO: 112 - DNA, 20 bp, artificial sequence
  sgRNA
gggcacactgaagaaaaact

SEQ ID NO: 113 - DNA, 20 bp, artificial sequence
  sgRNA
ggcacactgaagaaaaactg

SEQ ID NO: 114 - DNA, 20 bp, artificial sequence
  sgRNA
gcacactgaagaaaaactgg

SEQ ID NO: 115 - DNA, 20 bp, artificial sequence
  sgRNA
actgaagaaaaactggggga

SEQ ID NO: 116 - DNA, 20 bp, artificial sequence
  sgRNA
aactgggggaaggtgtatga

SEQ ID NO: 117 - DNA, 20 bp, artificial sequence
  sgRNA
actgggggaaggtgtatgaa

SEQ ID NO: 118 - DNA, 20 bp, artificial sequence
  sgRNA
atgaagggagctgcgagctg

SEQ ID NO: 119 - DNA, 20 bp, artificial sequence
  sgRNA
acatcaaaacattaatacaa

SEQ ID NO: 120 - DNA, 20 bp, artificial sequence
  sgRNA
attgtattaatgttttgatg

SEQ ID NO: 121 - DNA, 20 bp, artificial sequence
  sgRNA
tagggagagggtcggaggac

SEQ ID NO: 122 - DNA, 20 bp, artificial sequence
  sgRNA
gaagctagggagagggtcgg

SEQ ID NO: 123 - DNA, 20 bp, artificial sequence
  sgRNA
tgggaagctagggagagggt

SEQ ID NO: 124 - DNA, 20 bp, artificial sequence
  sgRNA
ggtctgggaagctagggaga

SEQ ID NO: 125 - DNA, 20 bp, artificial sequence
  sgRNA
gggtctgggaagctagggag

SEQ ID NO: 126 - DNA, 20 bp, artificial sequence
  sgRNA
gcaaggggtctgggaagcta

SEQ ID NO: 127 - DNA, 20 bp, artificial sequence
  sgRNA
agcaaggggtctgggaagct

SEQ ID NO: 128 - DNA, 20 bp, artificial sequence
  sgRNA
gggacaagagcaaggggtct

SEQ ID NO: 129 - DNA, 20 bp, artificial sequence
  sgRNA
tgggacaagagcaaggggtc

SEQ ID NO: 130 - DNA, 20 bp, artificial sequence
  sgRNA
caaagtgggacaagagcaag

SEQ ID NO: 131 - DNA, 20 bp, artificial sequence
  sgRNA
gcaaagtgggacaagagcaa

SEQ ID NO: 132 - DNA, 20 bp, artificial sequence
  sgRNA
ggcaaagtgggacaagagca

SEQ ID NO: 133 - DNA, 20 bp, artificial sequence
  sgRNA
caactcatgggtggcaaagt

SEQ ID NO: 134 - DNA, 20 bp, artificial sequence
  sgRNA
tcaactcatgggtggcaaag

SEQ ID NO: 135 - DNA, 20 bp, artificial sequence
  sgRNA
ccattaaatcaactcatggg

SEQ ID NO: 136 - DNA, 20 bp, artificial sequence
  sgRNA
aagccattaaatcaactcat

SEQ ID NO: 137 - DNA, 20 bp, artificial sequence
  sgRNA
taagccattaaatcaactca

SEQ ID NO: 138 - DNA, 20 bp, artificial sequence
  sgRNA
ccacccatgagttgatttaa

SEQ ID NO: 139 - DNA, 20 bp, artificial sequence
  sgRNA
cttaaatagtgctgaaatat

SEQ ID NO: 140 - DNA, 20 bp, artificial sequence
  sgRNA
aaatagtgctgaaatattgg

SEQ ID NO: 141 - DNA, 20 bp, artificial sequence
  sgRNA
ggctgagagtggaggcagat

SEQ ID NO: 142 - DNA, 20 bp, artificial sequence
  sgRNA
atctctgtggctgagagtgg

SEQ ID NO: 143 - DNA, 20 bp, artificial sequence
  sgRNA
gggatctctgtggctgagag

SEQ ID NO: 144 - DNA, 20 bp, artificial sequence
  sgRNA
ctccaaaaaagggatctctg

SEQ ID NO: 145 - DNA, 20 bp, artificial sequence
  sgRNA
agccacagagatcccttttt

SEQ ID NO: 146 - DNA, 20 bp, artificial sequence
  sgRNA
cgagtcatccctccaaaaaa

SEQ ID NO: 147 - DNA, 20 bp, artificial sequence
  sgRNA
tcgagtcatccctccaaaaa

SEQ ID NO: 148 - DNA, 20 bp, artificial sequence
  sgRNA
cacagagatcccttttttgg

SEQ ID NO: 149 - DNA, 20 bp, artificial sequence
  sgRNA
acagagatcccttttttgga

SEQ ID NO: 150 - DNA, 20 bp, artificial sequence
  sgRNA
tcgagatgaagatgatgatg

SEQ ID NO: 151 - DNA, 20 bp, artificial sequence
  sgRNA
gatgaggaagaagaagaaga

SEQ ID NO: 152 - DNA, 20 bp, artificial sequence
  sgRNA
atgaggaagaagaagaagaa

SEQ ID NO: 153 - DNA, 20 bp, artificial sequence
  sgRNA
tgaggaagaagaagaagaag

SEQ ID NO: 154 - DNA, 20 bp, artificial sequence
  sgRNA
gaggaagaagaagaagaagg

SEQ ID NO: 155 - DNA, 20 bp, artificial sequence
  sgRNA
aagaagaagaagggggctca

SEQ ID NO: 156 - DNA, 20 bp, artificial sequence
  sgRNA
agaagaagaagggggctcat

SEQ ID NO: 157 - DNA, 20 bp, artificial sequence
  sgRNA
gaagaagaagggggctcatg

SEQ ID NO: 158 - DNA, 20 bp, artificial sequence
  sgRNA
gaagggggctcatggggccg

SEQ ID NO: 159 - DNA, 20 bp, artificial sequence
  sgRNA
aagggggctcatggggccgt

SEQ ID NO: 160 - DNA, 20 bp, artificial sequence
  sgRNA
tatggaaccttgggttccca

SEQ ID NO: 161 - DNA, 20 bp, artificial sequence
  sgRNA
catggggccgtgggaaccca

SEQ ID NO: 162 - DNA, 20 bp, artificial sequence
  sgRNA
gctgaggactatggaacctt

SEQ ID NO: 163 - DNA, 20 bp, artificial sequence
  sgRNA
tgctgaggactatggaacct

SEQ ID NO: 164 - DNA, 20 bp, artificial sequence
  sgRNA
caggggggtgctgaggacta

SEQ ID NO: 165 - DNA, 20 bp, artificial sequence
  sgRNA
aattcctcaggggggtgctg

SEQ ID NO: 166 - DNA, 20 bp, artificial sequence
  sgRNA
tagtcctcagcacccccctg

SEQ ID NO: 167 - DNA, 20 bp, artificial sequence
  sgRNA
cgaagccaaattcctcaggg

SEQ ID NO: 168 - DNA, 20 bp, artificial sequence
  sgRNA
ccgaagccaaattcctcagg

SEQ ID NO: 169 - DNA, 20 bp, artificial sequence
  sgRNA
gccgaagccaaattcctcag

SEQ ID NO: 170 - DNA, 20 bp, artificial sequence
  sgRNA
agccgaagccaaattcctca

SEQ ID NO: 171 - DNA, 20 bp, artificial sequence
  sgRNA
aagccgaagccaaattcctc

SEQ ID NO: 172 - DNA, 20 bp, artificial sequence
  sgRNA
cagcacccccctgaggaatt

SEQ ID NO: 173 - DNA, 20 bp, artificial sequence
  sgRNA
ccccctgaggaatttggctt

SEQ ID NO: 174 - DNA, 20 bp, artificial sequence
  sgRNA
ttcggcttcagcttcagccc

SEQ ID NO: 175 - DNA, 20 bp, artificial sequence
  sgRNA
ggcttcagcttcagcccagg

SEQ ID NO: 176 - DNA, 20 bp, artificial sequence
  sgRNA
ttcagcttcagcccaggagg

SEQ ID NO: 177 - DNA, 20 bp, artificial sequence
  sgRNA
ggaaacgtatccctcctcct

SEQ ID NO: 178 - DNA, 20 bp, artificial sequence
  sgRNA
tcagcttcagcccaggagga

SEQ ID NO: 179 - DNA, 20 bp, artificial sequence
  sgRNA
tggaaacgtatccctcctcc

SEQ ID NO: 180 - DNA, 20 bp, artificial sequence
  sgRNA
catcaaagccgaagttatcg

SEQ ID NO: 181 - DNA, 20 bp, artificial sequence
  sgRNA
atacgtttccacgataactt

SEQ ID NO: 182 - DNA, 20 bp, artificial sequence
  sgRNA
tgctattgaaatctcgtact

SEQ ID NO: 183 - DNA, 20 bp, artificial sequence
  sgRNA
caatagcatcttcagcgata

SEQ ID NO: 184 - DNA, 20 bp, artificial sequence
  sgRNA
aatagcatcttcagcgatat

SEQ ID NO: 185 - DNA, 20 bp, artificial sequence
  sgRNA
atagcatcttcagcgatatg

SEQ ID NO: 186 - DNA, 20 bp, artificial sequence
  sgRNA
tagcatcttcagcgatatgg

SEQ ID NO: 187 - DNA, 20 bp, artificial sequence
  sgRNA
tcttcagcgatatgggggcc

SEQ ID NO: 188 - DNA, 20 bp, artificial sequence
  sgRNA
aggatgggaaggcaaggtcc

SEQ ID NO: 189 - DNA, 20 bp, artificial sequence
  sgRNA
accaggaggatgggaaggca

SEQ ID NO: 190 - DNA, 20 bp, artificial sequence
  sgRNA
cacacaccaggaggatggga

SEQ ID NO: 191 - DNA, 20 bp, artificial sequence
  sgRNA
aagccacacaccaggaggat

SEQ ID NO: 192 - DNA, 20 bp, artificial sequence
  sgRNA
accttgccttcccatcctcc

SEQ ID NO: 193 - DNA, 20 bp, artificial sequence
  sgRNA
aaagccacacaccaggagga

SEQ ID NO: 194 - DNA, 20 bp, artificial sequence
  sgRNA
agggaaagccacacaccagg

SEQ ID NO: 195 - DNA, 20 bp, artificial sequence
  sgRNA
cttcccatcctcctggtgtg

SEQ ID NO: 196 - DNA, 20 bp, artificial sequence
  sgRNA
cttagggaaagccacacacc

SEQ ID NO: 197 - DNA, 20 bp, artificial sequence
  sgRNA
ctggtgtgtggctttcccta

SEQ ID NO: 198 - DNA, 20 bp, artificial sequence
  sgRNA
tggtgtgtggctttccctaa

SEQ ID NO: 199 - DNA, 20 bp, artificial sequence
  sgRNA
ggtgtgtggctttccctaag

SEQ ID NO: 200 - DNA, 20 bp, artificial sequence
  sgRNA
aaaccacaggttgcccctta

SEQ ID NO: 201 - DNA, 20 bp, artificial sequence
  sgRNA
gaaaccacaggttgcccctt

SEQ ID NO: 202 - DNA, 20 bp, artificial sequence
  sgRNA
tttccctaaggggcaacctg

SEQ ID NO: 203 - DNA, 20 bp, artificial sequence
  sgRNA
accaacccaccagaaaccac

SEQ ID NO: 204 - DNA, 20 bp, artificial sequence
  sgRNA
aaggggcaacctgtggtttc

SEQ ID NO: 205 - DNA, 20 bp, artificial sequence
  sgRNA
gggcaacctgtggtttctgg

SEQ ID NO: 206 - DNA, 20 bp, artificial sequence
  sgRNA
ggcaacctgtggtttctggt

SEQ ID NO: 207 - DNA, 20 bp, artificial sequence
  sgRNA
acctgtggtttctggtgggt

SEQ ID NO: 208 - DNA, 20 bp, artificial sequence
  sgRNA
tgtggtttctggtgggttgg

SEQ ID NO: 209 - DNA, 20 bp, artificial sequence
  sgRNA
gtggtttctggtgggttggt

SEQ ID NO: 210 - DNA, 20 bp, artificial sequence
  sgRNA
gggtgaaataaagagcctgc

SEQ ID NO: 211 - DNA, 20 bp, artificial sequence
  sgRNA
ggtgaaataaagagcctgca

SEQ ID NO: 212 - DNA, 20 bp, artificial sequence
  sgRNA
atcccccagctactccctgc

SEQ ID NO: 213 - DNA, 20 bp, artificial sequence
  sgRNA
aagagcctgcagggagtagc

SEQ ID NO: 214 - DNA, 20 bp, artificial sequence
  sgRNA
agagcctgcagggagtagct

SEQ ID NO: 215 - DNA, 20 bp, artificial sequence
  sgRNA
gagcctgcagggagtagctg

SEQ ID NO: 216 - DNA, 20 bp, artificial sequence
  sgRNA
agcctgcagggagtagctgg

SEQ ID NO: 217 - DNA, 20 bp, artificial sequence
  sgRNA
tgcagggagtagctggggga

SEQ ID NO: 218 - DNA, 20 bp, artificial sequence
  sgRNA
gcagggagtagctgggggat

SEQ ID NO: 219 - DNA, 20 bp, artificial sequence
  sgRNA
gctgggatgggaaaggactt

SEQ ID NO: 220 - DNA, 20 bp, artificial sequence
  sgRNA
tgctgggatgggaaaggact

SEQ ID NO: 221 - DNA, 20 bp, artificial sequence
  sgRNA
ggtgtttgctgggatgggaa

SEQ ID NO: 222 - DNA, 20 bp, artificial sequence
  sgRNA
tggcaggtgtttgctgggat

SEQ ID NO: 223 - DNA, 20 bp, artificial sequence
  sgRNA
gtggcaggtgtttgctggga

SEQ ID NO: 224 - DNA, 20 bp, artificial sequence
  sgRNA
aaaggtggcaggtgtttgct

SEQ ID NO: 225 - DNA, 20 bp, artificial sequence
  sgRNA
gaaaggtggcaggtgtttgc

SEQ ID NO: 226 - DNA, 20 bp, artificial sequence
  sgRNA
aagttctgcagaaaggtggc

SEQ ID NO: 227 - DNA, 20 bp, artificial sequence
  sgRNA
ctggaagttctgcagaaagg

SEQ ID NO: 228 - DNA, 20 bp, artificial sequence
  sgRNA
gacctggaagttctgcagaa

SEQ ID NO: 229 - DNA, 20 bp, artificial sequence
  sgRNA
cacctttctgcagaacttcc

SEQ ID NO: 230 - DNA, 20 bp, artificial sequence
  sgRNA
ggtgtctctgactcaggacc

SEQ ID NO: 231 - DNA, 20 bp, artificial sequence
  sgRNA
tcaccaggtgtctctgactc

SEQ ID NO: 232 - DNA, 20 bp, artificial sequence
  sgRNA
ggtcctgagtcagagacacc

SEQ ID NO: 233 - DNA, 20 bp, artificial sequence
  sgRNA
ccctcccgtagtctctcacc

SEQ ID NO: 234 - DNA, 20 bp, artificial sequence
  sgRNA
agacacctggtgagagacta

SEQ ID NO: 235 - DNA, 20 bp, artificial sequence
  sgRNA
gacacctggtgagagactac

SEQ ID NO: 236 - DNA, 20 bp, artificial sequence
  sgRNA
acctggtgagagactacggg

SEQ ID NO: 237 - DNA, 20 bp, artificial sequence
  sgRNA
cctggtgagagactacggga

SEQ ID NO: 238 - DNA, 20 bp, artificial sequence
  sgRNA
tacgggagggacagacactt

SEQ ID NO: 239 - DNA, 20 bp, artificial sequence
  sgRNA
acgggagggacagacacttc

SEQ ID NO: 240 - DNA, 20 bp, artificial sequence
  sgRNA
atcctgggctggtgactatc

SEQ ID NO: 241 - DNA, 20 bp, artificial sequence
  sgRNA
atccagatagtcaccagccc

SEQ ID NO: 242 - DNA, 20 bp, artificial sequence
  sgRNA
cccccccaaagatcctgggc

SEQ ID NO: 243 - DNA, 20 bp, artificial sequence
  sgRNA
aagacccccccaaagatcct

SEQ ID NO: 244 - DNA, 20 bp, artificial sequence
  sgRNA
caagacccccccaaagatcc

SEQ ID NO: 245 - DNA, 20 bp, artificial sequence
  sgRNA
agtcaccagcccaggatctt

SEQ ID NO: 246 - DNA, 20 bp, artificial sequence
  sgRNA
gtcaccagcccaggatcttt

SEQ ID NO: 247 - DNA, 20 bp, artificial sequence
  sgRNA
tcaccagcccaggatctttg

SEQ ID NO: 248 - DNA, 20 bp, artificial sequence
  sgRNA
caccagcccaggatctttgg

SEQ ID NO: 249 - DNA, 20 bp, artificial sequence
  sgRNA
accagcccaggatctttggg

SEQ ID NO: 250 - DNA, 20 bp, artificial sequence
  sgRNA
ccagcccaggatctttgggg

SEQ ID NO: 251 - DNA, 20 bp, artificial sequence
  sgRNA
caggatctttgggggggtct

SEQ ID NO: 252 - DNA, 20 bp, artificial sequence
  sgRNA
ccagtctggtgctggttggg

SEQ ID NO: 253 - DNA, 20 bp, artificial sequence
  sgRNA
cccagtctggtgctggttgg

SEQ ID NO: 254 - DNA, 20 bp, artificial sequence
  sgRNA
ccccagtctggtgctggttg

SEQ ID NO: 255 - DNA, 20 bp, artificial sequence
  sgRNA
gccccagtctggtgctggtt

SEQ ID NO: 256 - DNA, 20 bp, artificial sequence
  sgRNA
agccccagtctggtgctggt

SEQ ID NO: 257 - DNA, 20 bp, artificial sequence
  sgRNA
tgggagccccagtctggtgc

SEQ ID NO: 258 - DNA, 20 bp, artificial sequence
  sgRNA
ccccccaaccagcaccagac

SEQ ID NO: 259 - DNA, 20 bp, artificial sequence
  sgRNA
cccccaaccagcaccagact

SEQ ID NO: 260 - DNA, 20 bp, artificial sequence
  sgRNA
ccccaaccagcaccagactg

SEQ ID NO: 261 - DNA, 20 bp, artificial sequence
  sgRNA
ggcctctgggagccccagtc

SEQ ID NO: 262 - DNA, 20 bp, artificial sequence
  sgRNA
caccagactggggctcccag

SEQ ID NO: 263 - DNA, 20 bp, artificial sequence
  sgRNA
caccctatgaaatggcctct

SEQ ID NO: 264 - DNA, 20 bp, artificial sequence
  sgRNA
tcaccctatgaaatggcctc

SEQ ID NO: 265 - DNA, 20 bp, artificial sequence
  sgRNA
gctcccagaggccatttcat

SEQ ID NO: 266 - DNA, 20 bp, artificial sequence
  sgRNA
gggatactcaccctatgaaa

SEQ ID NO: 267 - DNA, 20 bp, artificial sequence
  sgRNA
ctcccagaggccatttcata

SEQ ID NO: 268 - DNA, 20 bp, artificial sequence
  sgRNA
catagggtgagtatcccatc

SEQ ID NO: 269 - DNA, 20 bp, artificial sequence
  sgRNA
ctctcacttcaggaccagat

SEQ ID NO: 270 - DNA, 20 bp, artificial sequence
  sgRNA
gctctcacttcaggaccaga

SEQ ID NO: 271 - DNA, 20 bp, artificial sequence
  sgRNA
ctctcacaagctctcacttc

SEQ ID NO: 272 - DNA, 20 bp, artificial sequence
  sgRNA
cagtctttgcactttattag

SEQ ID NO: 273 - DNA, 20 bp, artificial sequence
  sgRNA
cactaataaagtgcaaagac

SEQ ID NO: 274 - DNA, 20 bp, artificial sequence
  sgRNA
ataaagtgcaaagactggct

SEQ ID NO: 275 - DNA, 20 bp, artificial sequence
  sgRNA
gtgcaaagactggctaggtg

SEQ ID NO: 276 - DNA, 20 bp, artificial sequence
  sgRNA
caaagactggctaggtgcgg

SEQ ID NO: 277 - DNA, 20 bp, artificial sequence
  sgRNA
tcccaaagtgctgggattac

SEQ ID NO: 278 - DNA, 20 bp, artificial sequence
  sgRNA
cctcggcctcccaaagtgct

SEQ ID NO: 279 - DNA, 20 bp, artificial sequence
  sgRNA
cgcctgtaatcccagcactt

SEQ ID NO: 280 - DNA, 20 bp, artificial sequence
  sgRNA
acctcggcctcccaaagtgc

SEQ ID NO: 281 - DNA, 20 bp, artificial sequence
  sgRNA
gcctgtaatcccagcacttt

SEQ ID NO: 282 - DNA, 20 bp, artificial sequence
  sgRNA
tgtaatcccagcactttggg

SEQ ID NO: 283 - DNA, 20 bp, artificial sequence
  sgRNA
cccagcactttgggaggccg

SEQ ID NO: 284 - DNA, 20 bp, artificial sequence
  sgRNA
agcactttgggaggccgagg

SEQ ID NO: 285 - DNA, 20 bp, artificial sequence
  sgRNA
gcactttgggaggccgaggt

SEQ ID NO: 286 - DNA, 20 bp, artificial sequence
  sgRNA
ctctggtgatctgcccacct

SEQ ID NO: 287 - DNA, 20 bp, artificial sequence
  sgRNA
cgaggtgggcagatcaccag

SEQ ID NO: 288 - DNA, 20 bp, artificial sequence
  sgRNA
tgggcagatcaccagaggtc

SEQ ID NO: 289 - DNA, 20 bp, artificial sequence
  sgRNA
ggtctccaactcctgacctc

SEQ ID NO: 290 - DNA, 20 bp, artificial sequence
  sgRNA
gatcaccagaggtcaggagt

SEQ ID NO: 291 - DNA, 20 bp, artificial sequence
  sgRNA
tcaggagttggagaccagcc

SEQ ID NO: 292 - DNA, 20 bp, artificial sequence
  sgRNA
tttcaccatgttgaccaggc

SEQ ID NO: 293 - DNA, 20 bp, artificial sequence
  sgRNA
ggggtttcaccatgttgacc

SEQ ID NO: 294 - DNA, 20 bp, artificial sequence
  sgRNA
ggagaccagcctggtcaaca

SEQ ID NO: 295 - DNA, 20 bp, artificial sequence
  sgRNA
ttgtatttttagtagacacg

SEQ ID NO: 296 - DNA, 20 bp, artificial sequence
  sgRNA
tttgtatttttagtagacac

SEQ ID NO: 297 - DNA, 20 bp, artificial sequence
  sgRNA
ttttgtatttttagtagaca

SEQ ID NO: 298 - DNA, 20 bp, artificial sequence
  sgRNA
taaaaatacaaaaaattagc

SEQ ID NO: 299 - DNA, 20 bp, artificial sequence
  sgRNA
aaaaatacaaaaaattagcc

SEQ ID NO: 300 - DNA, 20 bp, artificial sequence
  sgRNA
tacaaaaaattagccgggca

SEQ ID NO: 301 - DNA, 20 bp, artificial sequence
  sgRNA
caggcacctgccaccatgcc

SEQ ID NO: 302 - DNA, 20 bp, artificial sequence
  sgRNA
aaaaaattagccgggcatgg

SEQ ID NO: 303 - DNA, 20 bp, artificial sequence
  sgRNA
aattagccgggcatggtggc

SEQ ID NO: 304 - DNA, 20 bp, artificial sequence
  sgRNA
tcctgagtagctggcattac

SEQ ID NO: 305 - DNA, 20 bp, artificial sequence
  sgRNA
gcctcagcctcctgagtagc

SEQ ID NO: 306 - DNA, 20 bp, artificial sequence
  sgRNA
gcctgtaatgccagctactc

SEQ ID NO: 307 - DNA, 20 bp, artificial sequence
  sgRNA
tgtaatgccagctactcagg

SEQ ID NO: 308 - DNA, 20 bp, artificial sequence
  sgRNA
gccagctactcaggaggctg

SEQ ID NO: 309 - DNA, 20 bp, artificial sequence
  sgRNA
gctactcaggaggctgaggc

SEQ ID NO: 310 - DNA, 20 bp, artificial sequence
  sgRNA
ggaggctgaggcaggagaat

SEQ ID NO: 311 - DNA, 20 bp, artificial sequence
  sgRNA
caggagaattggttgaaccc

SEQ ID NO: 312 - DNA, 20 bp, artificial sequence
  sgRNA
gagaattggttgaacccagg

SEQ ID NO: 313 - DNA, 20 bp, artificial sequence
  sgRNA
aattggttgaacccaggagg

SEQ ID NO: 314 - DNA, 20 bp, artificial sequence
  sgRNA
agatggagtctccacctcct

SEQ ID NO: 315 - DNA, 20 bp, artificial sequence
  sgRNA
gagatggagtctccacctcc

SEQ ID NO: 316 - DNA, 20 bp, artificial sequence
  sgRNA
gtctcaaacaatttttgaga

SEQ ID NO: 317 - DNA, 20 bp, artificial sequence
  sgRNA
ctgggcaacagagcaaggct

SEQ ID NO: 318 - DNA, 20 bp, artificial sequence
  sgRNA
cctgggcaacagagcaaggc

SEQ ID NO: 319 - DNA, 20 bp, artificial sequence
  sgRNA
acagcctgggcaacagagca

SEQ ID NO: 320 - DNA, 20 bp, artificial sequence
  sgRNA
ccagccttgctctgttgccc

SEQ ID NO: 321 - DNA, 20 bp, artificial sequence
  sgRNA
gtgccacggcactacagcct

SEQ ID NO: 322 - DNA, 20 bp, artificial sequence
  sgRNA
tgtgccacggcactacagcc

SEQ ID NO: 323 - DNA, 20 bp, artificial sequence
  sgRNA
ttgcccaggctgtagtgccg

SEQ ID NO: 324 - DNA, 20 bp, artificial sequence
  sgRNA
agtgagctgagattgtgcca

SEQ ID NO: 325 - DNA, 20 bp, artificial sequence
  sgRNA
cacttgaacctgggaattgg

SEQ ID NO: 326 - DNA, 20 bp, artificial sequence
  sgRNA
cactgcaacctccaattccc

SEQ ID NO: 327 - DNA, 20 bp, artificial sequence
  sgRNA
aatcacttgaacctgggaat

SEQ ID NO: 328 - DNA, 20 bp, artificial sequence
  sgRNA
caggagaatcacttgaacct

SEQ ID NO: 329 - DNA, 20 bp, artificial sequence
  sgRNA
gcaggagaatcacttgaacc

SEQ ID NO: 330 - DNA, 20 bp, artificial sequence
  sgRNA
gctactcaggaggctgaggc

SEQ ID NO: 331 - DNA, 20 bp, artificial sequence
  sgRNA
cccagctactcaggaggctg

SEQ ID NO: 332 - DNA, 20 bp, artificial sequence
  sgRNA
tgtaatcccagctactcagg

SEQ ID NO: 333 - DNA, 20 bp, artificial sequence
  sgRNA
gactgtaatcccagctactc

SEQ ID NO: 334 - DNA, 20 bp, artificial sequence
  sgRNA
gcctcagcctcctgagtagc

SEQ ID NO: 335 - DNA, 20 bp, artificial sequence
  sgRNA
cctcagcctcctgagtagct

SEQ ID NO: 336 - DNA, 20 bp, artificial sequence
  sgRNA
aaattagctgggcgtttggc

SEQ ID NO: 337 - DNA, 20 bp, artificial sequence
  sgRNA
acaaaaattagctgggcgtt

SEQ ID NO: 338 - DNA, 20 bp, artificial sequence
  sgRNA
taaaaacacaaaaattagct

SEQ ID NO: 339 - DNA, 20 bp, artificial sequence
  sgRNA
ctaaaaacacaaaaattagc

SEQ ID NO: 340 - DNA, 20 bp, artificial sequence
  sgRNA
ttttgtgtttttagtagaga

SEQ ID NO: 341 - DNA, 20 bp, artificial sequence
  sgRNA
gagatggcgtttcaccgtgt

SEQ ID NO: 342 - DNA, 20 bp, artificial sequence
  sgRNA
caaaagcagcctggccaaca

SEQ ID NO: 343 - DNA, 20 bp, artificial sequence
  sgRNA
ggcgtttcaccgtgttggcc

SEQ ID NO: 344 - DNA, 20 bp, artificial sequence
  sgRNA
tcaggagctcaaaagcagcc

SEQ ID NO: 345 - DNA, 20 bp, artificial sequence
  sgRNA
gcttttgagctcctgacctc

SEQ ID NO: 346 - DNA, 20 bp, artificial sequence
  sgRNA
tgggtggatcacctgaggtc

SEQ ID NO: 347 - DNA, 20 bp, artificial sequence
  sgRNA
cgaggtgggtggatcacctg

SEQ ID NO: 348 - DNA, 20 bp, artificial sequence
  sgRNA
ctttgggaggccgaggtggg

SEQ ID NO: 349 - DNA, 20 bp, artificial sequence
  sgRNA
ctcaggtgatccacccacct

SEQ ID NO: 350 - DNA, 20 bp, artificial sequence
  sgRNA
gcactttgggaggccgaggt

SEQ ID NO: 351 - DNA, 20 bp, artificial sequence
  sgRNA
agcactttgggaggccgagg

SEQ ID NO: 352 - DNA, 20 bp, artificial sequence
  sgRNA
tccagcactttgggaggccg

SEQ ID NO: 353 - DNA, 20 bp, artificial sequence
  sgRNA
tgtaattccagcactttggg

SEQ ID NO: 354 - DNA, 20 bp, artificial sequence
  sgRNA
acttgtaattccagcacttt

SEQ ID NO: 355 - DNA, 20 bp, artificial sequence
  sgRNA
acctcggcctcccaaagtgc

SEQ ID NO: 356 - DNA, 20 bp, artificial sequence
  sgRNA
cacttgtaattccagcactt

SEQ ID NO: 357 - DNA, 20 bp, artificial sequence
  sgRNA
caatctttggccaggcatga

SEQ ID NO: 358 - DNA, 20 bp, artificial sequence
  sgRNA
caagtgtgagccatcatgcc

SEQ ID NO: 359 - DNA, 20 bp, artificial sequence
  sgRNA
aagaattgcaatctttggcc

SEQ ID NO: 360 - DNA, 20 bp, artificial sequence
  sgRNA
caaacaagaattgcaatctt

SEQ ID NO: 361 - DNA, 20 bp, artificial sequence
  sgRNA
ttgtttgaatctgatagcct

SEQ ID NO: 362 - DNA, 20 bp, artificial sequence
  sgRNA
tgtttgaatctgatagcctt

SEQ ID NO: 363 - DNA, 20 bp, artificial sequence
  sgRNA
tgaatctgatagccttgggt

SEQ ID NO: 364 - DNA, 20 bp, artificial sequence
  sgRNA
gggcttaggattccaaccca

SEQ ID NO: 365 - DNA, 20 bp, artificial sequence
  sgRNA
aaacactaaatggagggctt

SEQ ID NO: 366 - DNA, 20 bp, artificial sequence
  sgRNA
aacagaaaacactaaatgga

SEQ ID NO: 367 - DNA, 20 bp, artificial sequence
  sgRNA
aaacagaaaacactaaatgg

SEQ ID NO: 368 - DNA, 20 bp, artificial sequence
  sgRNA
agaaaacagaaaacactaaa

SEQ ID NO: 369 - DNA, 20 bp, artificial sequence
  sgRNA
tgttttctatattaagcttg

SEQ ID NO: 370 - DNA, 20 bp, artificial sequence
  sgRNA
gttttctatattaagcttgt

SEQ ID NO: 371 - DNA, 20 bp, artificial sequence
  sgRNA
taagcttgtgggattttctt

SEQ ID NO: 372 - DNA, 20 bp, artificial sequence
  sgRNA
aagcttgtgggattttcttt

SEQ ID NO: 373 - DNA, 20 bp, artificial sequence
  sgRNA
agcttgtgggattttctttg

SEQ ID NO: 374 - DNA, 20 bp, artificial sequence
  sgRNA
gcttgtgggattttctttgg

SEQ ID NO: 375 - DNA, 20 bp, artificial sequence
  sgRNA
cttgtgggattttctttggg

SEQ ID NO: 376 - DNA, 20 bp, artificial sequence
  sgRNA
ggattttctttggggggaga

SEQ ID NO: 377 - DNA, 20 bp, artificial sequence
  sgRNA
gattttctttggggggagat

SEQ ID NO: 378 - DNA, 20 bp, artificial sequence
  sgRNA
caaaaacaaaaaaacaccac

SEQ ID NO: 379 - DNA, 20 bp, artificial sequence
  sgRNA
ccaagaattatctagaccag

SEQ ID NO: 380 - DNA, 20 bp, artificial sequence
  sgRNA
ccactggtctagataattct

SEQ ID NO: 381 - DNA, 20 bp, artificial sequence
  sgRNA
gtctagataattcttggata

SEQ ID NO: 382 - DNA, 20 bp, artificial sequence
  sgRNA
agataattcttggataaggc

SEQ ID NO: 383 - DNA, 20 bp, artificial sequence
  sgRNA
taaggcaggattgtgcacag

SEQ ID NO: 384 - DNA, 20 bp, artificial sequence
  sgRNA
caggattgtgcacagaggat

SEQ ID NO: 385 - DNA, 20 bp, artificial sequence
  sgRNA
ggataggaatatatcagttc

SEQ ID NO: 386 - DNA, 20 bp, artificial sequence
  sgRNA
atcagttcaggaagtctttc

SEQ ID NO: 387 - DNA, 20 bp, artificial sequence
  sgRNA
caggaagtctttctggtaga

SEQ ID NO: 388 - DNA, 20 bp, artificial sequence
  sgRNA
gaaggatacataaaacagcc

SEQ ID NO: 389 - DNA, 20 bp, artificial sequence
  sgRNA
gatacataaaacagccagga

SEQ ID NO: 390 - DNA, 20 bp, artificial sequence
  sgRNA
cttatttacacactccttcc

SEQ ID NO: 391 - DNA, 20 bp, artificial sequence
  sgRNA
caggaaggagtgtgtaaata

SEQ ID NO: 392 - DNA, 20 bp, artificial sequence
  sgRNA
gtaaataaggctattctgaa

SEQ ID NO: 393 - DNA, 20 bp, artificial sequence
  sgRNA
gaatggaattatctcttctg

SEQ ID NO: 394 - DNA, 20 bp, artificial sequence
  sgRNA
ggaattatctcttctgtgga

SEQ ID NO: 395 - DNA, 20 bp, artificial sequence
  sgRNA
gaattatctcttctgtggaa

SEQ ID NO: 396 - DNA, 20 bp, artificial sequence
  sgRNA
aattatctcttctgtggaag

SEQ ID NO: 397 - DNA, 20 bp, artificial sequence
  sgRNA
attatctcttctgtggaagg

SEQ ID NO: 398 - DNA, 20 bp, artificial sequence
  sgRNA
tcttctgtggaagggggttt

SEQ ID NO: 399 - DNA, 20 bp, artificial sequence
  sgRNA
tggaagggggttttggagct

SEQ ID NO: 400 - DNA, 20 bp, artificial sequence
  sgRNA
ggaagggggttttggagctc

SEQ ID NO: 401 - DNA, 20 bp, artificial sequence
  sgRNA
tggagctcgggagtagtttg

SEQ ID NO: 402 - DNA, 20 bp, artificial sequence
  sgRNA
cttccaatctgaaatttgaa

SEQ ID NO: 403 - DNA, 20 bp, artificial sequence
  sgRNA
tgacctttcaaatttcagat

SEQ ID NO: 404 - DNA, 20 bp, artificial sequence
  sgRNA
ctttcaaatttcagattgga

SEQ ID NO: 405 - DNA, 20 bp, artificial sequence
  sgRNA
aggagtcttttcacttacta

SEQ ID NO: 406 - DNA, 20 bp, artificial sequence
  sgRNA
ttctgcagtttgatgatgta

SEQ ID NO: 407 - DNA, 20 bp, artificial sequence
  sgRNA
gtttgatgatgtatggccta

SEQ ID NO: 408 - DNA, 20 bp, artificial sequence
  sgRNA
gttctaggatgggggtccat

SEQ ID NO: 409 - DNA, 20 bp, artificial sequence
  sgRNA
cctctctggttctaggatgg

SEQ ID NO: 410 - DNA, 20 bp, artificial sequence
  sgRNA
tcctctctggttctaggatg

SEQ ID NO: 411 - DNA, 20 bp, artificial sequence
  sgRNA
gtcctctctggttctaggat

SEQ ID NO: 412 - DNA, 20 bp, artificial sequence
  sgRNA
tgtcctctctggttctagga

SEQ ID NO: 413 - DNA, 20 bp, artificial sequence
  sgRNA
ccattgtcctctctggttct

SEQ ID NO: 414 - DNA, 20 bp, artificial sequence
  sgRNA
cccccatcctagaaccagag

SEQ ID NO: 415 - DNA, 20 bp, artificial sequence
  sgRNA
agacttaccattgtcctctc

SEQ ID NO: 416 - DNA, 20 bp, artificial sequence
  sgRNA
cctagaaccagagaggacaa

SEQ ID NO: 417 - DNA, 20 bp, artificial sequence
  sgRNA
agagaggacaatggtaagtc

SEQ ID NO: 418 - DNA, 20 bp, artificial sequence
  sgRNA
gaggacaatggtaagtctgg

SEQ ID NO: 419 - DNA, 20 bp, artificial sequence
  sgRNA
acaatggtaagtctggagga

SEQ ID NO: 420 - DNA, 20 bp, artificial sequence
  sgRNA
caatggtaagtctggaggaa

SEQ ID NO: 421 - DNA, 20 bp, artificial sequence
  sgRNA
aatggtaagtctggaggaag

SEQ ID NO: 422 - DNA, 20 bp, artificial sequence
  sgRNA
tcagaagaataacaaaaggc

SEQ ID NO: 423 - DNA, 20 bp, artificial sequence
  sgRNA
aacttcagaagaataacaaa

SEQ ID NO: 424 - DNA, 20 bp, artificial sequence
  sgRNA
acaggaagaaacttcaggga

SEQ ID NO: 425 - DNA, 20 bp, artificial sequence
  sgRNA
tacaggaagaaacttcaggg

SEQ ID NO: 426 - DNA, 20 bp, artificial sequence
  sgRNA
gtgtacaggaagaaacttca

SEQ ID NO: 427 - DNA, 20 bp, artificial sequence
  sgRNA
agtgtacaggaagaaacttc

SEQ ID NO: 428 - DNA, 20 bp, artificial sequence
  sgRNA
aaaaaaggagacaagtgtac

SEQ ID NO: 429 - DNA, 20 bp, artificial sequence
  sgRNA
gaaagagtccaaaggaaaaa

SEQ ID NO: 430 - DNA, 20 bp, artificial sequence
  sgRNA
acttgtctccttttttcctt

SEQ ID NO: 431 - DNA, 20 bp, artificial sequence
  sgRNA
gcaggagagaaagagtccaa

SEQ ID NO: 432 - DNA, 20 bp, artificial sequence
  sgRNA
gagcagagagatgaagaagc

SEQ ID NO: 433 - DNA, 20 bp, artificial sequence
  sgRNA
gaaacctgggaatcaagatc

SEQ ID NO: 434 - DNA, 20 bp, artificial sequence
  sgRNA
tcttccagatcttgattccc

SEQ ID NO: 435 - DNA, 20 bp, artificial sequence
  sgRNA
aagaccctcctgggaaacct

SEQ ID NO: 436 - DNA, 20 bp, artificial sequence
  sgRNA
caagaccctcctgggaaacc

SEQ ID NO: 437 - DNA, 20 bp, artificial sequence
  sgRNA
tcttgattcccaggtttccc

SEQ ID NO: 438 - DNA, 20 bp, artificial sequence
  sgRNA
tgattcccaggtttcccagg

SEQ ID NO: 439 - DNA, 20 bp, artificial sequence
  sgRNA
gattcccaggtttcccagga

SEQ ID NO: 440 - DNA, 20 bp, artificial sequence
  sgRNA
aaccgggccaagaccctcct

SEQ ID NO: 441 - DNA, 20 bp, artificial sequence
  sgRNA
gaaccgggccaagaccctcc

SEQ ID NO: 442 - DNA, 20 bp, artificial sequence
  sgRNA
caggtttcccaggagggtct

SEQ ID NO: 443 - DNA, 20 bp, artificial sequence
  sgRNA
ttcccaggagggtcttggcc

SEQ ID NO: 444 - DNA, 20 bp, artificial sequence
  sgRNA
tgggctggggctgtagaacc

SEQ ID NO: 445 - DNA, 20 bp, artificial sequence
  sgRNA
ttgggctggggctgtagaac

SEQ ID NO: 446 - DNA, 20 bp, artificial sequence
  sgRNA
ttgaaataggatttgggctg

SEQ ID NO: 447 - DNA, 20 bp, artificial sequence
  sgRNA
cttgaaataggatttgggct

SEQ ID NO: 448 - DNA, 20 bp, artificial sequence
  sgRNA
tcttgaaataggatttgggc

SEQ ID NO: 449 - DNA, 20 bp, artificial sequence
  sgRNA
atgctcttgaaataggattt

SEQ ID NO: 450 - DNA, 20 bp, artificial sequence
  sgRNA
gatgctcttgaaataggatt

SEQ ID NO: 451 - DNA, 20 bp, artificial sequence
  sgRNA
cacagagatgctcttgaaat

SEQ ID NO: 452 - DNA, 20 bp, artificial sequence
  sgRNA
cccatctggtttagtgatct

SEQ ID NO: 453 - DNA, 20 bp, artificial sequence
  sgRNA
accaagatcactaaaccaga

SEQ ID NO: 454 - DNA, 20 bp, artificial sequence
  sgRNA
ccaagatcactaaaccagat

SEQ ID NO: 455 - DNA, 20 bp, artificial sequence
  sgRNA
caagatcactaaaccagatg

SEQ ID NO: 456 - DNA, 20 bp, artificial sequence
  sgRNA
ttctttcaactcaccccatc

SEQ ID NO: 457 - DNA, 20 bp, artificial sequence
  sgRNA
tggggtgagttgaaagaaag

SEQ ID NO: 458 - DNA, 20 bp, artificial sequence
  sgRNA
gagttgaaagaaagaggtaa

SEQ ID NO: 459 - DNA, 20 bp, artificial sequence
  sgRNA
gaaagaggtaaaggaaagta

SEQ ID NO: 460 - DNA, 20 bp, artificial sequence
  sgRNA
aggtaaaggaaagtatggcc

SEQ ID NO: 461 - DNA, 20 bp, artificial sequence
  sgRNA
ggtaaaggaaagtatggcca

SEQ ID NO: 462 - DNA, 20 bp, artificial sequence
  sgRNA
gtttcagggcattcgttccc

SEQ ID NO: 463 - DNA, 20 bp, artificial sequence
  sgRNA
gggaacgaatgccctgaaac

SEQ ID NO: 464 - DNA, 20 bp, artificial sequence
  sgRNA
ttacacagatccctgtttca

SEQ ID NO: 465 - DNA, 20 bp, artificial sequence
  sgRNA
ggaacgaatgccctgaaaca

SEQ ID NO: 466 - DNA, 20 bp, artificial sequence
  sgRNA
tttacacagatccctgtttc

SEQ ID NO: 467 - DNA, 20 bp, artificial sequence
  sgRNA
catattccgaatgttactaa

SEQ ID NO: 468 - DNA, 20 bp, artificial sequence
  sgRNA
gcataacctttagtaacatt

SEQ ID NO: 469 - DNA, 20 bp, artificial sequence
  sgRNA
ctttagtaacattcggaata

SEQ ID NO: 470 - DNA, 20 bp, artificial sequence
  sgRNA
tagtaacattcggaatatgg

SEQ ID NO: 471 - DNA, 20 bp, artificial sequence
  sgRNA
agtaacattcggaatatggt

SEQ ID NO: 472 - DNA, 20 bp, artificial sequence
  sgRNA
gtaacattcggaatatggtg

SEQ ID NO: 473 - DNA, 20 bp, artificial sequence
  sgRNA
ggacttctctttgtagatag

SEQ ID NO: 474 - DNA, 20 bp, artificial sequence
  sgRNA
cttctctttgtagatagtgg

SEQ ID NO: 475 - DNA, 20 bp, artificial sequence
  sgRNA
tgtagatagtggaggagcgc

SEQ ID NO: 476 - DNA, 20 bp, artificial sequence
  sgRNA
agtggaggagcgccggactg

SEQ ID NO: 477 - DNA, 20 bp, artificial sequence
  sgRNA
cctcactgtccaccacagtc

SEQ ID NO: 478 - DNA, 20 bp, artificial sequence
  sgRNA
ggaggagcgccggactgtgg

SEQ ID NO: 479 - DNA, 20 bp, artificial sequence
  sgRNA
ccggactgtggtggacagtg

SEQ ID NO: 480 - DNA, 20 bp, artificial sequence
  sgRNA
cggactgtggtggacagtga

SEQ ID NO: 481 - DNA, 20 bp, artificial sequence
  sgRNA
ctgtggtggacagtgagggc

SEQ ID NO: 482 - DNA, 20 bp, artificial sequence
  sgRNA
gggttactgtagtctctgtc

SEQ ID NO: 483 - DNA, 20 bp, artificial sequence
  sgRNA
actgctatctgcttcgtgtc

SEQ ID NO: 484 - DNA, 20 bp, artificial sequence
  sgRNA
gactgctatctgcttcgtgt

SEQ ID NO: 485 - DNA, 20 bp, artificial sequence
  sgRNA
acgaagcagatagcagtcct

SEQ ID NO: 486 - DNA, 20 bp, artificial sequence
  sgRNA
cgaagcagatagcagtccta

SEQ ID NO: 487 - DNA, 20 bp, artificial sequence
  sgRNA
gaagcagatagcagtcctag

SEQ ID NO: 488 - DNA, 20 bp, artificial sequence
  sgRNA
gcagatagcagtcctagggg

SEQ ID NO: 489 - DNA, 20 bp, artificial sequence
  sgRNA
tcttttaacttaccacccct

SEQ ID NO: 490 - DNA, 20 bp, artificial sequence
  sgRNA
ggtggtaagttaaaagacaa

SEQ ID NO: 491 - DNA, 20 bp, artificial sequence
  sgRNA
gtggtaagttaaaagacaaa

SEQ ID NO: 492 - DNA, 20 bp, artificial sequence
  sgRNA
tggtaagttaaaagacaaag

SEQ ID NO: 493 - DNA, 20 bp, artificial sequence
  sgRNA
gggttcatctcaagattcct

SEQ ID NO: 494 - DNA, 20 bp, artificial sequence
  sgRNA
ggttcatctcaagattcctt

SEQ ID NO: 495 - DNA, 20 bp, artificial sequence
  sgRNA
gttcatctcaagattccttg

SEQ ID NO: 496 - DNA, 20 bp, artificial sequence
  sgRNA
atctcaagattccttgggga

SEQ ID NO: 497 - DNA, 20 bp, artificial sequence
  sgRNA
agtaagatttcccttcccca

SEQ ID NO: 498 - DNA, 20 bp, artificial sequence
  sgRNA
tctcaagattccttggggaa

SEQ ID NO: 499 - DNA, 20 bp, artificial sequence
  sgRNA
taggcagaagcaaaggacaa

SEQ ID NO: 500 - DNA, 20 bp, artificial sequence
  sgRNA
ctaggcagaagcaaaggaca

SEQ ID NO: 501 - DNA, 20 bp, artificial sequence
  sgRNA
aagagactaggcagaagcaa

SEQ ID NO: 502 - DNA, 20 bp, artificial sequence
  sgRNA
taggctaaatgaaagagact

SEQ ID NO: 503 - DNA, 20 bp, artificial sequence
  sgRNA
agaaagtcatacacgtaaat

SEQ ID NO: 504 - DNA, 20 bp, artificial sequence
  sgRNA
tcttggtgattctggatcta

SEQ ID NO: 505 - DNA, 20 bp, artificial sequence
  sgRNA
gctggaggtcttggtgattc

SEQ ID NO: 506 - DNA, 20 bp, artificial sequence
  sgRNA
tcatccagggctggaggtct

SEQ ID NO: 507 - DNA, 20 bp, artificial sequence
  sgRNA
aaggcatcatccagggctgg

SEQ ID NO: 508 - DNA, 20 bp, artificial sequence
  sgRNA
atcaccaagacctccagccc

SEQ ID NO: 509 - DNA, 20 bp, artificial sequence
  sgRNA
gaaaaggcatcatccagggc

SEQ ID NO: 510 - DNA, 20 bp, artificial sequence
  sgRNA
gatggaaaaggcatcatcca

SEQ ID NO: 511 - DNA, 20 bp, artificial sequence
  sgRNA
ggatggaaaaggcatcatcc

SEQ ID NO: 512 - DNA, 20 bp, artificial sequence
  sgRNA
gaataagtccaggatggaaa

SEQ ID NO: 513 - DNA, 20 bp, artificial sequence
  sgRNA
ggatgatgccttttccatcc

SEQ ID NO: 514 - DNA, 20 bp, artificial sequence
  sgRNA
tcccaggaataagtccagga

SEQ ID NO: 515 - DNA, 20 bp, artificial sequence
  sgRNA
aacgtcccaggaataagtcc

SEQ ID NO: 516 - DNA, 20 bp, artificial sequence
  sgRNA
ttccatcctggacttattcc

SEQ ID NO: 517 - DNA, 20 bp, artificial sequence
  sgRNA
tccatcctggacttattcct

SEQ ID NO: 518 - DNA, 20 bp, artificial sequence
  sgRNA
gggaccggaaccaacgtccc

SEQ ID NO: 519 - DNA, 20 bp, artificial sequence
  sgRNA
tggacttattcctgggacgt

SEQ ID NO: 520 - DNA, 20 bp, artificial sequence
  sgRNA
tattcctgggacgttggttc

SEQ ID NO: 521 - DNA, 20 bp, artificial sequence
  sgRNA
tgggacgttggttccggtcc

SEQ ID NO: 522 - DNA, 20 bp, artificial sequence
  sgRNA
gttaacaaggctaccgggac

SEQ ID NO: 523 - DNA, 20 bp, artificial sequence
  sgRNA
tgagggttaacaaggctacc

SEQ ID NO: 524 - DNA, 20 bp, artificial sequence
  sgRNA
ctgagggttaacaaggctac

SEQ ID NO: 525 - DNA, 20 bp, artificial sequence
  sgRNA
aaggcctctgagggttaaca

SEQ ID NO: 526 - DNA, 20 bp, artificial sequence
  sgRNA
gtagccttgttaaccctcag

SEQ ID NO: 527 - DNA, 20 bp, artificial sequence
  sgRNA
aaggacttgaaggcctctga

SEQ ID NO: 528 - DNA, 20 bp, artificial sequence
  sgRNA
aaaggacttgaaggcctctg

SEQ ID NO: 529 - DNA, 20 bp, artificial sequence
  sgRNA
gagaggtggaaaggacttga

SEQ ID NO: 530 - DNA, 20 bp, artificial sequence
  sgRNA
gcaatgggtgagaggtggaa

SEQ ID NO: 531 - DNA, 20 bp, artificial sequence
  sgRNA
ggtgggcaatgggtgagagg

SEQ ID NO: 532 - DNA, 20 bp, artificial sequence
  sgRNA
aatggtgggcaatgggtgag

SEQ ID NO: 533 - DNA, 20 bp, artificial sequence
  sgRNA
gcttattaatggtgggcaat

SEQ ID NO: 534 - DNA, 20 bp, artificial sequence
  sgRNA
agcttattaatggtgggcaa

SEQ ID NO: 535 - DNA, 20 bp, artificial sequence
  sgRNA
aagctaagcttattaatggt

SEQ ID NO: 536 - DNA, 20 bp, artificial sequence
  sgRNA
gaagctaagcttattaatgg

SEQ ID NO: 537 - DNA, 20 bp, artificial sequence
  sgRNA
agagaagctaagcttattaa

SEQ ID NO: 538 - DNA, 20 bp, artificial sequence
  sgRNA
ttagcttctcttgccacctc

SEQ ID NO: 539 - DNA, 20 bp, artificial sequence
  sgRNA
tagcttctcttgccacctca

SEQ ID NO: 540 - DNA, 20 bp, artificial sequence
  sgRNA
agcttctcttgccacctcag

SEQ ID NO: 541 - DNA, 20 bp, artificial sequence
  sgRNA
acatatccaagcccctgagg

SEQ ID NO: 542 - DNA, 20 bp, artificial sequence
  sgRNA
tccacatatccaagcccctg

SEQ ID NO: 543 - DNA, 20 bp, artificial sequence
  sgRNA
ctcttgccacctcaggggct

SEQ ID NO: 544 - DNA, 20 bp, artificial sequence
  sgRNA
acctcaggggcttggatatg

SEQ ID NO: 545 - DNA, 20 bp, artificial sequence
  sgRNA
ggatatgtggaatagtgaac

SEQ ID NO: 546 - DNA, 20 bp, artificial sequence
  sgRNA
gatatgtggaatagtgaact

SEQ ID NO: 547 - DNA, 20 bp, artificial sequence
  sgRNA
atatgtggaatagtgaactg

SEQ ID NO: 548 - DNA, 20 bp, artificial sequence
  sgRNA
gggtgagtgacaaactgaca

SEQ ID NO: 549 - DNA, 20 bp, artificial sequence
  sgRNA
aaggttttattggtcagttt

SEQ ID NO: 550 - DNA, 20 bp, artificial sequence
  sgRNA
aaaggttttattggtcagtt

SEQ ID NO: 551 - DNA, 20 bp, artificial sequence
  sgRNA
agcataaataaaggttttat

SEQ ID NO: 552 - DNA, 20 bp, artificial sequence
  sgRNA
gctgagggctatggaacctt

SEQ ID NO: 553 - DNA, 20 bp, artificial sequence
  sgRNA
gctgaggactatggaacctt

SEQ ID NO: 554 - DNA, 20 bp, artificial sequence
  sgRNA
ctccctcccaggatcctctc

SEQ ID NO: 555 - DNA, 21 bp, artificial sequence
  primer
caccttatattcccagggccg

SEQ ID NO: 556 - DNA, 21 bp, artificial sequence
  primer
cctaggacgcaccattctcac

SEQ ID NO: 557 - DNA, 22 bp, artificial sequence
  primer
tccagcctgggaaacatgagag

SEQ ID NO: 558 - DNA, 22 bp, artificial sequence
  primer
actactcccgagctccaaaacc

SEQ ID NO: 559 - DNA, 21 bp, artificial sequence
  primer
caccttatattcccagggccg

SEQ ID NO: 560 - DNA, 23 bp, artificial sequence
  primer
ccatgagttgatttaatggctta

SEQ ID NO: 561 - DNA, 24 bp, artificial sequence
  primer
acatcgcccaggtcagtcaaaaag

SEQ ID NO: 562 - DNA, 22 bp, artificial sequence
  primer
aaacactaaatggagggcttag

SEQ ID NO: 563 - DNA, 45 bp, artificial sequence
  primer
gaggactatggaacctaggattgccgcgtccccatgagccccctt

SEQ ID NO: 564 - DNA, 45 bp, artificial sequence
  primer
aagggggctcatggggacgcggcaatcctaggttccatagtcctc

SEQ ID NO: 565 - DNA, 2406 bp, artificial sequence
  repair template
acatcgcccaggtcagtcaaaaagaacgcccgagtaaggagcgaggtggcttctgctgtgaggctggccagccccgcgggtggggtggttgagggacgccctcaagccggtccatttgtgcggctgggctgccctctggcggctttatccgggtgccatccagagtcaaaccctcgaaatcgcttttcgtactgagttggtctgcagaaagaagaacagatttaggaggaaggcggtcataggaaactgaaagtgcgtcacgcccactcccgtcacggaaactggtctctgaaaggtggggtaaagataaagcctttcaaatttgaggaagaccttcggtcccgcctccatttcacgtccggcttaccgtcgtttacgacagtgtcaggatcgcgggcttgctttccggtagcgtgggctgacgcctcgctcaatttctcacagggctgcgcaggtttcccccgtctgcgaatggaccactggaggggttcaaaggttcgcgtcccagtacgggaatgagcctctttgatctcttccggggctttttcggctttcctggacctcggaggtgagagtaggtccggctcggacaagggtgggggtcgtctgaggggagcttgacccctacgtcttatttttggaaaaacatcctctgtcccactccttcaactcctgcagagaggacagaagtcgcaacattgaacactcaccccgccacagtaaccaaggcggtcattaagaggagaaacagcaaactaagcctttctccaacctggggtgatgcaacagggacccgggcggggaagaccgtgagggtctggggaataagacagtgagcaagtgagcaggaccttgggagagagaggagggactggggcacactgaagaaaaactgggggaaggtgtatgaagggagctgcgagctgaggtctgactttgattaaaaaaaaaaaaaaaaaaaaagaactgtcagccattgtattaatgttttgatgtggcagccagtcctccgaccctctccctagcttcccagaccccttgctcttgtcccactttgccacccatgagttgatttaatggcttaaatagtgctgaaatattggtggccaatctgcctccactctcagccacagagatcccttttttggagggatgactcgagatgaagatgatgatgaggaagaagaagaagaagggggctcatggggacgcggcaatcctaggttccatagtcctcagcacccccctgaggaatttggcttcggcttcagcttcagcccaggaggagggatacgtttccacgataacttcggctttgatgacctagtacgagatttcaatagcatcttcagcgatatgggggcctggaccttgccttcccatcctcctggtgtgtggctttccctaaggggcaacctgtggtttctggtgggttggtgggtgaaataaagagcctgcagggagtagctgggggatgggaagtgtgagaagactgatgatttcagagagattaatagagcccaagtcctttcccatcccagcaaacacctgccacctttctgcagaacttccaggtcctgagtcagagacacctggtgagagactacgggagggacagacacttcgggactcaatgcttaagtatccagatagtcaccagcccaggatctttgggggggtcttggagagtgatgcaagaagtgaatccccccaaccagcaccagactggggctcccagaggccatttcatagggtgagtatcccatctggtcctgaagtgagagcttgtgagagaccactaataaagtgcaaagactggctaggtgcggtggctcacgcctgtaatcccagcactttgggaggccgaggtgggcagatcaccagaggtcaggagttggagaccagcctggtcaacatggtgaaaccccgtgtctactaaaaatacaaaaaattagccgggcatggtggcaggtgcctgtaatgccagctactcaggaggctgaggcaggagaattggttgaacccaggaggtggagactccatctcaaaaattgtttgagacccagccttgctctgttgcccaggctgtagtgccgtggcacaatctcagctcactgcaacctccaattcccaggttcaagtgattctcctgcctcagcctcctgagtagctgggattacagtcgcctgccaaacgcccagctaatttttgtgtttttagtagagatggcgtttcaccgtgttggccaggctgcttttgagctcctgacctcaggtgatccacccacctcggcctcccaaagtgctggaattacaagtgtgagccatcatgcctggccaaagattgcaattcttgtttgaatctgatagccttgggttggaatcctaagccctccatttagtgttt